European Patent Application EP 4 640 710 A1, published October 29, 2025. Title: Monoclonal antibody specifically binding to claudin-18.2 and uses thereof. Applicant: Y-Biologics Inc. Application KR. The sequence listing filed with the application follows.

SEQUENCE LISTING (16 sequences)

SEQ ID NO: 1 - protein, 8 aa, synthetic construct
GFTFSSYA

SEQ ID NO: 2 - protein, 8 aa, synthetic construct
ISGSGGST

SEQ ID NO: 3 - protein, 13 aa, synthetic construct
AKEGVWWLRYFDH

SEQ ID NO: 4 - protein, 120 aa, synthetic construct
QVQLVESGGGLVQPGGSLRLSCAASGFTFSSYAMSWVRQAPGKGLEWVAAISGSGGSTYFADSVRGRFTISRDNPQSTLYLQMNSLRAEDTAVYYCAKEGVWWLRYFDHWGQGTPITVSS

SEQ ID NO: 5 - protein, 9 aa, synthetic construct
SNDVGGYTY

SEQ ID NO: 6 - protein, 10 aa, synthetic construct
SSYAGSYTWV

SEQ ID NO: 7 - protein, 110 aa, synthetic construct
QSALTQPRSVSGSPGQSVTISCTGTSNDVGGYTYVSWYQQHPGKAPKLMIYDVSKRPSGVPDRFSGSKSGNTASLTISGLQAEDEADYYCSSYAGSYTWVFGGGTKLTVL

SEQ ID NO: 8 - protein, 13 aa, synthetic construct
ARGLGYYYYGMDV

SEQ ID NO: 9 - protein, 120 aa, synthetic construct
QMQLVESGGGLVQPGGSLRLSCAASGFTFSSYAMSWVRQAPGKGLEWVSAISGSGGSTYYADSVKGRFTISRDNSKNTLYLQMNSLRAEDTAVYYCARGLGYYYYGMDVWGQGTTVTVSS

SEQ ID NO: 10 - protein, 6 aa, synthetic construct
QTVSSW

SEQ ID NO: 11 - protein, 9 aa, synthetic construct
QQYHSFPPT

SEQ ID NO: 12 - protein, 107 aa, synthetic construct
DIQMTQSPSSLSASVGDRVTITCRASQTVSSWLAWYQQKPGKAPKLLIYAASSLQSGVPSRFSGSGSGTEFTLTISSLQPEDFGTYYCQQYHSFPPTFGGGTKVGIK

SEQ ID NO: 13 - protein, 12 aa, synthetic construct
ARGAASSYYFDY

SEQ ID NO: 14 - protein, 119 aa, synthetic construct
QVQLVQSGGGLVQPGGSLRLSCAASGFTFSSYAMSWVRQAPGKGLEWVSAISGSGGSTYYADSVKGRFTISRDNSKNTLYLQMNSLRAEDTAVYYCARGAASSYYFDYWGLGTTVTVSS

SEQ ID NO: 15 - protein, 6 aa, synthetic construct
AGVRNY

SEQ ID NO: 16 - protein, 107 aa, synthetic construct
DIQMTQSPSSLAAYVGDTVTITCRASAGVRNYLAWVQQKPGKAPRSLIYGAFKLQSGVPSRFSGSGSGTEFTLTISSLQPEDFGTYYCQQYHSFPPTFGGGTKVDIK